European Patent Application EP 4 289 494 A1, published December 13, 2023. Title: 一种制备多肽的细胞裂解液分离设备、系统及其应用. Applicant: 重庆誉颜制药有限公司. The sequence listing filed with the application follows.

SEQUENCE LISTING (1 sequence)

SEQ ID NO: 1 - protein, 1524 aa, Artificial Sequence
MSPILGYWKIKGLVQPTRLLLEYLEEKYEEHLYERDEGDKWRNKKFELGLEFPNLPYYIDGDVKLTQSMAIIRYIADKHNMLGGCPKERAEISMLEGAVLDIRYGVSRIAYSKDFETLKVDFLSKLPEMLKMFEDRLCHKTYLNGDHVTHPDFMLYDALDVVLYMDPMCLDAFPKLVCFKKRIEAIPQIDKYLKSSKYIAWPLQGWQATFGGGDHPPKSDLEVLFQGPLGSMPFVNKQFNYKDPVNGVDIAYIKIPNAGQMQPVKAFKIHNKIWVIPERDTFTNPEEGDLNPPPEAKQVPVSYYDSTYLSTDNEKDNYLKGVTKLFERIYSTDLGRMLLTSIVRGIPFWGGSTIDTELKVIDTNCINVIQPDGSYRSEELNLVIIGPSADIIQFECKSFGHEVLNLTRNGYGSTQYIRFSPDFTFGFEESLEVDTNPLLGAGKFATDPAVTLAHELIHAGHRLYGIAINPNRVFKVNTNAYYEMSGLEVSFEELRTFGGHDAKFIDSLQENEFRLYYYNKFKDIASTLNKAKSIVGTTASLQYMKNVFKEKYLLSEDTSGKFSVDKLKFDKLYKMLTEIYTEDNFVKFFKVLNRKTYLNFDKAVFKINIVPKVNYTIYDGFNLRNTNLAANFNGQNTEINNMNFTKLKNFTGLFEFYKLLCVRGIITSLEVLFQGPALNDLCIKVNNWDLFFSPSEDNFTNDLNKGEEITSDTNIEAAEENISLDLIQQYYLTFNFDNEPENISIENLSSDIIGQLELMPNIERFPNGKKYELDKYTMFHYLRAQEFEHGKSRIALTNSVNEALLNPSRVYTFFSSDYVKKVNKATEAAMFLGWVEQLVYDFTDETSEVSTTDKIADITIIIPYIGPALNIGNMLYKDDFVGALIFSGAVILLEFIPEIAIPVLGTFALVSYIANKVLTVQTIDNALSKRNEKWDEVYKYIVTNWLAKVNTQIDLIRKKMKEALENQAEATKAIINYQYNQYTEEEKNNINFNIDDLSSKLNESINKAMININKFLNQCSVSYLMNSMIPYGVKRLEDFDASLKDALLKYIYDNRGTLIGQVDRLKDKVNNTLSTDIPFQLSKYVDNQRLLSTFTEYIKNIINTSILNLRYESNHLIDLSRYASKINIGSKVNFDPIDKNQIQLFNLESSKIEVILKNAIVYNSMYENFSTSFWIRIPKYFNSISLNNEYTIINCMENNSGWKVSLNYGEIIWTLQDTQEIKQRVVFKYSQMINISDYINRWIFVTITNNRLNNSKIYINGRLIDQKPISNLGNIHASNNIMFKLDGCRDTHRYIWIKYFNLFDKELNEKEIKDLYDNQSNSGILKDFWGDYLQYDKPYYMLNLYDPNKYVDVNNVGIRGYMYLKGPRGSVMTTNIYLNSSLYRGTKFIIKKYASGNKDNIVRNNDRVYINVVVKNKEYRLATNASQAGVEKILSALEIPDVGNLSQVVVMKSKNDQGITNKCKMNLQDNNGNDIGFIGFHQFNNIAKLVASNWYNRQIERSSRTLGCSWEFIPVDDGWGERPL